European Patent Specification EP 3 313 880 B1, published August 6, 2025. Title: ANTIBODIES TO CD40. Applicant: Bristol-Myers Squibb Company. The sequence listing filed with the application follows.

SEQUENCE LISTING (78 sequences)

SEQ ID NO: 1 - protein, 277 aa, Homo sapiens
  SIGNAL (1)..(20)
  PEPTIDE (21)..(277)
  DOMAIN (21)..(193): extracellular domain
  DOMAIN (194)..(215): transmembrane domain
  DOMAIN (216)..(277): intracellular domain
MVRLPLQCVLWGCLLTAVHPEPPTACREKQYLINSQCCSLCQPGQKLVSDCTEFTETECLPCGESEFLDTWNRETHCHQHKYCDPNLGLRVQQKGTSETDTICTCEEGWHCTSEACESCVLHRSCSPGFGVKQIATGVSDTICEPCPVGFFSNVSSAFEKCHPWTSCETKDLVVQQAGTNKTDVVCGPQDRLRALVVIPIIFGILFAILLVLVFIKKVAKKPTNKAPHPKQEPQEINFPDDLPGSNTAAPVQETLHGCQPVTQEDGKESRISVQERQ

SEQ ID NO: 2 - protein, 261 aa, Homo sapiens
MIETYNQTSPRSAATGLPISMKIFMYLLTVFLITQMIGSALFAVYLHRRLDKIEDERNLHEDFVFMKTIQRCNTGERSLSLLNCEEIKSQFEGFVKDIMLNKEETKKENSFEMQKGDQNPQIAAHVISEASSKTTSVLQWAEKGYYTMSNNLVTLENGKQLTVKRQGLYYIYAQVTFCSNREASSQAPFIASLCLKSPGRFERILLRAANTHSSAKPCGQQSIHLGGVFELQPGASVFVNVTDPSQVSHGTGFTSFGLLKL

SEQ ID NO: 3 - protein, 448 aa, Artificial Sequence
  chimeric antibody with mouse variable domain, human constant domain
  DOMAIN (1)..(119): variable domain
  MISC_FEATURE (31)..(35): CDRH1
  MISC_FEATURE (50)..(66): CDRH2
  MISC_FEATURE (99)..(108): CDRH3
EVQLQQSGPELEKPGASVKMSCKASGYSFTGYNMNWVKQSNGKSLEWIGNIDPYYGNTNYNQKFKGKATLTVDKSSSTAYLQLKSLTSEDSAVYYCARLGLQLYAMDYWGQGTSVTVSSASTKGPSVFPLAPSSKSTSGGTAALGCLVKDYFPEPVTVSWNSGALTSGVHTFPAVLQSSGLYSLSSVVTVPSSSLGTQTYICNVNHKPSNTKVDKRVEPKSCDKTHTCPPCPAPELLGGPSVFLFPPKPKDTLMISRTPEVTCVVVDVSHEDPEVKFNWYVDGVEVHNAKTKPREEQYNSTYRVVSVLTVLHQDWLNGKEYKCKVSNKALPAPIEKTISKAKGQPREPQVYTLPPSREEMTKNQVSLTCLVKGFYPSDIAVEWESNGQPENNYKTTPPVLDSDGSFFLYSKLTVDKSRWQQGNVFSCSVMHEALHNHYTQKSLSLSPG

SEQ ID NO: 4 - protein, 219 aa, Artificial Sequence
  chimeric antibody with mouse variable domain and human constant domain
  DOMAIN (1)..(112): variable domain
  MISC_FEATURE (24)..(39): CDRL1
  MISC_FEATURE (55)..(61): CDRL2
  MISC_FEATURE (94)..(102): CDRL3
DVVMTQTPLSLPVSLGDQASISCRSSQSLVHSNGNTYLHWYLQKPGQSPNLLIYKLTNRFFGVPDRFSGSGSGTDFTLKISRVEAEDLGVYFCSQSIHVPWTFGGGTKLEIKRTVAAPSVFIFPPSDEQLKSGTASVVCLLNNFYPREAKVQWKVDNALQSGNSQESVTEQDSKDSTYSLSSTLTLSKADYEKHKVYACEVTHQGLSSPVTKSFNRGEC

SEQ ID NO: 5 - protein, 448 aa, Artificial Sequence
  humanized antibody with mouse CDRs and human framework and constant regions
  DOMAIN (1)..(119): variable domain
  MISC_FEATURE (31)..(35): CDRH1
  MISC_FEATURE (50)..(66): CDRH2
  MISC_FEATURE (99)..(108): CDRH3
QVQLVQSGAEVKKPGASVKVSCKASGYTFTGYNMNWVRQAPGQGLEWMGNIDPYYGNTNYNQKFKGRVTMTTDTSTSTAYMELRSLRSDDTAVYYCARLGLQLYAMDYWGQGTTVTVSSASTKGPSVFPLAPSSKSTSGGTAALGCLVKDYFPEPVTVSWNSGALTSGVHTFPAVLQSSGLYSLSSVVTVPSSSLGTQTYICNVNHKPSNTKVDKRVEPKSCDKTHTCPPCPAPELLGGPSVFLFPPKPKDTLMISRTPEVTCVVVDVSHEDPEVKFNWYVDGVEVHNAKTKPREEQYNSTYRVVSVLTVLHQDWLNGKEYKCKVSNKALPAPIEKTISKAKGQPREPQVYTLPPSREEMTKNQVSLTCLVKGFYPSDIAVEWESNGQPENNYKTTPPVLDSDGSFFLYSKLTVDKSRWQQGNVFSCSVMHEALHNHYTQKSLSLSPG

SEQ ID NO: 6 - protein, 219 aa, Artificial Sequence
  humanized antibody with mouse CDRs and human framework and constant regions
  DOMAIN (1)..(112): variable domain
  MISC_FEATURE (24)..(39): CDRL1
  MISC_FEATURE (55)..(61): CDRL2
  MISC_FEATURE (94)..(102): CDRL3
DIVMTQTPLSLPVTPGEPASISCRSSQSLVHSNGNTYLHWYLQKPGQSPQLLIYKLTNRFFGVPDRFSGSGSGTDFTLKISRVEAEDVGVYYCSQSIHVPWTFGGGTKVEIKRTVAAPSVFIFPPSDEQLKSGTASVVCLLNNFYPREAKVQWKVDNALQSGNSQESVTEQDSKDSTYSLSSTLTLSKADYEKHKVYACEVTHQGLSSPVTKSFNRGEC

SEQ ID NO: 7 - protein, 448 aa, Artificial Sequence; identical to SEQ ID NO: 5
  humanized antibody with mouse CDRs and human framework and constant regions
  DOMAIN (1)..(119): variable domain
  MISC_FEATURE (31)..(35): CDRH1
  MISC_FEATURE (50)..(66): CDRH2
  MISC_FEATURE (99)..(108): CDRH3

SEQ ID NO: 8 - protein, 448 aa, Artificial Sequence
  humanized antibody with mouse CDRs and human framework and constant regions
  DOMAIN (1)..(119): variable domain
  MISC_FEATURE (31)..(35): CDRH1
  MISC_FEATURE (50)..(66): CDRH2
  MISC_FEATURE (99)..(108): CDRH3
QVQLVQSGAEVKKPGASVKVSCKASGYTFTGYNMNWVRQAPGQGLEWMGNIDPYYGNTNYNQKFKGRVTMTTDTSTSTAYMELRSLRSDDTAVYYCARLGLQLYAMDYWGQGTTVTVSSASTKGPSVFPLAPSSKSTSGGTAALGCLVKDYFPEPVTVSWNSGALTSGVHTFPAVLQSSGLYSLSSVVTVPSSSLGTQTYICNVNHKPSNTKVDKRVEPKSCDKTHTCPPCPAPELLGDDSVFLFPPKPKDTLMISRTPEVTCVVVDVSHEDGEVKFNWYVDGVEVHNAKTKPREEQYNSTYRVVSVLTVLHQDWLNGKEYKCKVSNKALPRPIEKTISKAKGQPREPQVYTLPPSREEMTKNQVSLTCLVKGFYPSDIAVEWESNGQPENNYKTTPPVLDSDGSFFLYSKLTVDKSRWQQGNVFSCSVMHEALHNHYTQKSLSLSPG

SEQ ID NO: 9 - protein, 219 aa, Artificial Sequence
  humanized antibody with mouse CDRs and human framework and constant regions
  DOMAIN (1)..(112): variable domain
  MISC_FEATURE (24)..(39): CDRL1
  MISC_FEATURE (55)..(61): CDRL2
  MISC_FEATURE (94)..(102): CDRL3
DIVMTQTPLSLPVTPGEPASISCRSSQSLVHSNANTYLHWYLQKPGQSPQLLIYKLTNRFFGVPDRFSGSGSGTDFTLKISRVEAEDVGVYYCSQSIHVPWTFGGGTKVEIKRTVAAPSVFIFPPSDEQLKSGTASVVCLLNNFYPREAKVQWKVDNALQSGNSQESVTEQDSKDSTYSLSSTLTLSKADYEKHKVYACEVTHQGLSSPVTKSFNRGEC

SEQ ID NO: 10 - protein, 448 aa, Artificial Sequence
  humanized antibody with mouse CDRs and human framework and constant regions
  DOMAIN (1)..(119): variable domain
  MISC_FEATURE (31)..(35): CDRH1
  MISC_FEATURE (50)..(66): CDRH2
  MISC_FEATURE (99)..(108): CDRH3
QVQLVQSGAEVKKPGASVKVSCKASGYTFTGYNMNWVRQAPGQGLEWMGNIDPYYGNTNYNQKFKGRVTMTTDTSTSTAYMELRSLRSDDTAVYYCARLGLQLYALDYWGQGTTVTVSSASTKGPSVFPLAPSSKSTSGGTAALGCLVKDYFPEPVTVSWNSGALTSGVHTFPAVLQSSGLYSLSSVVTVPSSSLGTQTYICNVNHKPSNTKVDKRVEPKSCDKTHTCPPCPAPELLGGPSVFLFPPKPKDTLMISRTPEVTCVVVDVSHEDPEVKFNWYVDGVEVHNAKTKPREEQYNSTYRVVSVLTVLHQDWLNGKEYKCKVSNKALPAPIEKTISKAKGQPREPQVYTLPPSREEMTKNQVSLTCLVKGFYPSDIAVEWESNGQPENNYKTTPPVLDSDGSFFLYSKLTVDKSRWQQGNVFSCSVMHEALHNHYTQKSLSLSPG

SEQ ID NO: 11 - protein, 219 aa, Artificial Sequence; identical to SEQ ID NO: 6
  humanized antibody with mouse CDRs and human framework and constant regions
  DOMAIN (1)..(112): variable domain
  MISC_FEATURE (24)..(39): CDRL1
  MISC_FEATURE (55)..(61): CDRL2
  MISC_FEATURE (94)..(102): CDRL3

SEQ ID NO: 12 - protein, 448 aa, Artificial Sequence; identical to SEQ ID NO: 10
  humanized antibody with mouse CDRs and human framework and constant regions
  DOMAIN (1)..(119): variable domain
  MISC_FEATURE (31)..(35): CDRH1
  MISC_FEATURE (50)..(66): CDRH2
  MISC_FEATURE (99)..(108): CDRH3

SEQ ID NO: 13 - protein, 448 aa, Artificial Sequence
  humanized antibody with mouse CDRs and human framework and constant regions
  DOMAIN (1)..(119): variable domain
  MISC_FEATURE (31)..(35): CDRH1
  MISC_FEATURE (50)..(66): CDRH2
  MISC_FEATURE (99)..(108): CDRH3
QVQLVQSGAEVKKPGASVKVSCKASGYTFTGYNMNWVRQAPGQGLEWMGNIDPYYGNTNYNQKFKGRVTMTTDTSTSTAYMELRSLRSDDTAVYYCARLGLQLYALDYWGQGTTVTVSSASTKGPSVFPLAPSSKSTSGGTAALGCLVKDYFPEPVTVSWNSGALTSGVHTFPAVLQSSGLYSLSSVVTVPSSSLGTQTYICNVNHKPSNTKVDKRVEPKSCDKTHTCPPCPAPELLGGDSVFLFPPKPKDTLMISRTPEVTCVVVDVSHEDPEVKFNWYVDGVEVHNAKTKPREEQYNSTYRVVSVLTVLHQDWLNGKEYKCKVSNKALPAPIEKTISKAKGQPREPQVYTLPPSREEMTKNQVSLTCLVKGFYPSDIAVEWESNGQPENNYKTTPPVLDSDGSFFLYSKLTVDKSRWQQGNVFSCSVMHEALHNHYTQKSLSLSPG

SEQ ID NO: 14 - protein, 448 aa, Artificial Sequence
  humanized antibody with mouse CDRs and human framework and constant regions
  DOMAIN (1)..(119): variable domain
  MISC_FEATURE (31)..(35): CDRH1
  MISC_FEATURE (50)..(66): CDRH2
  MISC_FEATURE (99)..(108): CDRH3
QVQLVQSGAEVKKPGASVKVSCKASGYTFTGYNMNWVRQAPGQGLEWMGNIDPYYGNTNYNQKFKGRVTMTTDTSTSTAYMELRSLRSDDTAVYYCARLGLQLYALDYWGQGTTVTVSSASTKGPSVFPLAPSSKSTSGGTAALGCLVKDYFPEPVTVSWNSGALTSGVHTFPAVLQSSGLYSLSSVVTVPSSSLGTQTYICNVNHKPSNTKVDKRVEPKSCDKTHTCPPCPAPELLGGPSVFLFPPKPKDTLMISRTPEVTCVVVDVEHEDPEVKFNWYVDGVEVHNAKTKPREEQYNSTYRVVSVLTVLHQDWLNGKEYKCKVSNKALPAPIEKTISKAKGQPREPQVYTLPPSREEMTKNQVSLTCLVKGFYPSDIAVEWESNGQPENNYKTTPPVLDSDGSFFLYSKLTVDKSRWQQGNVFSCSVMHEALHNHYTQKSLSLSPG

SEQ ID NO: 15 - protein, 448 aa, Artificial Sequence
  humanized antibody with mouse CDRs and human framework and constant regions
  DOMAIN (1)..(119): variable domain
  MISC_FEATURE (31)..(35): CDRH1
  MISC_FEATURE (50)..(66): CDRH2
  MISC_FEATURE (99)..(108): CDRH3
QVQLVQSGAEVKKPGASVKVSCKASGYTFTGYNMNWVRQAPGQGLEWMGNIDPYYGNTNYNQKFKGRVTMTTDTSTSTAYMELRSLRSDDTAVYYCARLGLQLYALDYWGQGTTVTVSSASTKGPSVFPLAPSSKSTSGGTAALGCLVKDYFPEPVTVSWNSGALTSGVHTFPAVLQSSGLYSLSSVVTVPSSSLGTQTYICNVNHKPSNTKVDKRVEPKSCDKTHTCPPCPAPELLGGPSVFLFPPKPKDTLMISRTPEVTCVVVDVEHEDPEVKFNWYVDGVEVHNAKTKPREEQYNSTYRVVSVLTVLHQDWLNGKEYKCKVSNKAFPAPIEKTISKAKGQPREPQVYTLPPSREEMTKNQVSLTCLVKGFYPSDIAVEWESNGQPENNYKTTPPVLDSDGSFFLYSKLTVDKSRWQQGNVFSCSVMHEALHNHYTQKSLSLSPG

SEQ ID NO: 16 - protein, 448 aa, Artificial Sequence
  humanized antibody with mouse CDRs and human framework and constant regions
  DOMAIN (1)..(119): variable domain
  MISC_FEATURE (31)..(35): CDRH1
  MISC_FEATURE (50)..(66): CDRH2
  MISC_FEATURE (99)..(108): CDRH3
QVQLVQSGAEVKKPGASVKVSCKASGYTFTGYNMNWVRQAPGQGLEWMGNIDPYYGNTNYNQKFKGRVTMTTDTSTSTAYMELRSLRSDDTAVYYCARLGLQLYALDYWGQGTTVTVSSASTKGPSVFPLAPSSKSTSGGTAALGCLVKDYFPEPVTVSWNSGALTSGVHTFPAVLQSSGLYSLSSVVTVPSSSLGTQTYICNVNHKPSNTKVDKRVEPKSCDKTHTCPPCPAPELLGGDSVFLFPPKPKDTLMISRTPEVTCVVVDVSHEDGEVKFNWYVDGVEVHNAKTKPREEQYNSTYRVVSVLTVLHQDWLNGKEYKCKVSNKALPAPIEKTISKAKGQPREPQVYTLPPSREEMTKNQVSLTCLVKGFYPSDIAVEWESNGQPENNYKTTPPVLDSDGSFFLYSKLTVDKSRWQQGNVFSCSVMHEALHNHYTQKSLSLSPG

SEQ ID NO: 17 - protein, 448 aa, Artificial Sequence
  humanized antibody with mouse CDRs and human framework and constant regions
QVQLVQSGAEVKKPGASVKVSCKASGYTFTGYNMNWVRQAPGQGLEWMGNIDPYYGNTNYNQKFKGRVTMTTDTSTSTAYMELRSLRSDDTAVYYCARLGLQLYALDYWGQGTTVTVSSASTKGPSVFPLAPSSKSTSGGTAALGCLVKDYFPEPVTVSWNSGALTSGVHTFPAVLQSSGLYSLSSVVTVPSSSLGTQTYICNVNHKPSNTKVDKRVEPKSCDKTHTCPPCPAPELLGGDSVFLFPPKPKDTLMISRTPEVTCVVVDVSHEEGEVKFNWYVDGVEVHNAKTKPREEQYNSTYRVVSVLTVLHQDWLNGKEYKCKVSNKALPAPIEKTISKAKGQPREPQVYTLPPSREEMTKNQVSLTCLVKGFYPSDIAVEWESNGQPENNYKTTPPVLDSDGSFFLYSKLTVDKSRWQQGNVFSCSVMHEALHNHYTQKSLSLSPG

SEQ ID NO: 18 - protein, 448 aa, Artificial Sequence
  humanized antibody with mouse CDRs and human framework and constant regions
  DOMAIN (1)..(119): variable domain
  MISC_FEATURE (31)..(35): CDRH1
  MISC_FEATURE (50)..(66): CDRH2
  MISC_FEATURE (99)..(108): CDRH3
QVQLVQSGAEVKKPGASVKVSCKASGYTFTGYNMNWVRQAPGQGLEWMGNIDPYYGNTNYNQKFKGRVTMTTDTSTSTAYMELRSLRSDDTAVYYCARLGLQLYALDYWGQGTTVTVSSASTKGPSVFPLAPSSKSTSGGTAALGCLVKDYFPEPVTVSWNSGALTSGVHTFPAVLQSSGLYSLSSVVTVPSSSLGTQTYICNVNHKPSNTKVDKRVEPKSCDKTHTCPPCPAPELLGDDSVFLFPPKPKDTLMISRTPEVTCVVVDVSDEDGEVKFNWYVDGVEVHNAKTKPREEQYNSTYRVVSVLTVLHQDWLNGKEYKCKVSNKALPAPIEKTISKAKGQPREPQVYTLPPSREEMTKNQVSLTCLVKGFYPSDIAVEWESNGQPENNYKTTPPVLDSDGSFFLYSKLTVDKSRWQQGNVFSCSVMHEALHNHYTQKSLSLSPG

SEQ ID NO: 19 - protein, 448 aa, Artificial Sequence
  humanized antibody with mouse CDRs and human framework and constant regions
  DOMAIN (1)..(119): variable domain
  MISC_FEATURE (31)..(35): CDRH1
  MISC_FEATURE (50)..(66): CDRH2
  MISC_FEATURE (99)..(108): CDRH3
QVQLVQSGAEVKKPGASVKVSCKASGYTFTGYNMNWVRQAPGQGLEWMGNIDPYYGNTNYNQKFKGRVTMTTDTSTSTAYMELRSLRSDDTAVYYCARLGLQLYALDYWGQGTTVTVSSASTKGPSVFPLAPSSKSTSGGTAALGCLVKDYFPEPVTVSWNSGALTSGVHTFPAVLQSSGLYSLSSVVTVPSSSLGTQTYICNVNHKPSNTKVDKRVEPKSCDKTHTCPPCPAPELLGDDSVFLFPPKPKDTLMISRTPEVTCVVVDVSHEDGEVKFNWYVDGVEVHNAKTKPREEQYNSTYRVVSVLTVLHQDWLNGKEYKCKVSNKALPRPIEKTISKAKGQPREPQVYTLPPSREEMTKNQVSLTCLVKGFYPSDIAVEWESNGQPENNYKTTPPVLDSDGSFFLYSKLTVDKSRWQQGNVFSCSVMHEALHNHYTQKSLSLSPG

SEQ ID NO: 20 - protein, 448 aa, Artificial Sequence
  humanized antibody with mouse CDRs and human framework and constant regions
QVQLVQSGAEVKKPGASVKVSCKASGYTFTGYNMNWVRQAPGQGLEWMGNIDPYYGNTNYNQKFKGRVTMTTDTSTSTAYMELRSLRSDDTAVYYCARLGLQLYALDYWGQGTTVTVSSASTKGPSVFPLAPSSKSTSGGTAALGCLVKDYFPEPVTVSWNSGALTSGVHTFPAVLQSSGLYSLSSVVTVPSSSLGTQTYICNVNHKPSNTKVDKRVEPKSCDKTHTCPPCPAPELLGDDSVFLFPPKPKDTLMISRTPEVTCVVVDVSHEEGEVKFNWYVDGVEVHNAKTKPREEQYNSTYRVVSVLTVLHQDWLNGKEYKCKVSNKALPRPIEKTISKAKGQPREPQVYTLPPSREEMTKNQVSLTCLVKGFYPSDIAVEWESNGQPENNYKTTPPVLDSDGSFFLYSKLTVDKSRWQQGNVFSCSVMHEALHNHYTQKSLSLSPG

SEQ ID NO: 21 - protein, 448 aa, Artificial Sequence
  humanized antibody with mouse CDRs and human framework and constant regions
  DOMAIN (1)..(119): variable domain
  MISC_FEATURE (31)..(35): CDRH1
  MISC_FEATURE (50)..(66): CDRH2
  MISC_FEATURE (99)..(108): CDRH3
QVQLVQSGAEVKKPGASVKVSCKASGYTFTGYNMNWVRQAPGQGLEWMGNIDPYYGNTNYNQKFKGRVTMTTDTSTSTAYMELRSLRSDDTAVYYCARLGLQLYALDYWGQGTTVTVSSASTKGPSVFPLAPSSKSTSGGTAALGCLVKDYFPEPVTVSWNSGALTSGVHTFPAVLQSSGLYSLSSVVTVPSSSLGTQTYICNVNHKPSNTKVDKRVEPKSCDKTHTCPPCPAPELLGDDSVFLFPPKPKDTLMISRTPEVTCVVVDVSDEDGEVKFNWYVDGVEVHNAKTKPREEQYNSTYRVVSVLTVLHQDWLNGKEYKCKVSNKALPRPIEKTISKAKGQPREPQVYTLPPSREEMTKNQVSLTCLVKGFYPSDIAVEWESNGQPENNYKTTPPVLDSDGSFFLYSKLTVDKSRWQQGNVFSCSVMHEALHNHYTQKSLSLSPG

SEQ ID NO: 22 - protein, 448 aa, Artificial Sequence
  humanized antibody with mouse CDRs and human framework and constant regions
  DOMAIN (1)..(119): variable domain
  MISC_FEATURE (31)..(35): CDRH1
  MISC_FEATURE (50)..(66): CDRH2
  MISC_FEATURE (99)..(108): CDRH3
QVQLVQSGAEVKKPGASVKVSCKASGYTFTGYNMNWVRQAPGQGLEWMGNIDPYYGNTNYNQKFKGRVTMTTDTSTSTAYMELRSLRSDDTAVYYCARLGLQLYALDYWGQGTTVTVSSASTKGPSVFPLAPSSKSTSGGTAALGCLVKDYFPEPVTVSWNSGALTSGVHTFPAVLQSSGLYSLSSVVTVPSSSLGTQTYICNVNHKPSNTKVDKRVEPKSCDKTHTCPPCPAPDLLGDDSVFLFPPKPKDTLMISRTPEVTCVVVDVSDEDGEVKFNWYVDGVEVHNAKTKPREEQYNSTYRVVSVLTVLHQDWLNGKEYKCKVSNKALPRPIEKTISKAKGQPREPQVYTLPPSREEMTKNQVSLTCLVKGFYPSDIAVEWESNGQPENNYKTTPPVLDSDGSFFLYSKLTVDKSRWQQGNVFSCSVMHEALHNHYTQKSLSLSPG

SEQ ID NO: 23 - protein, 446 aa, Artificial Sequence
  chimeric antibody with mouse variable domain and human constant domain
  DOMAIN (1)..(117): variable domain
  MISC_FEATURE (31)..(35): CDRH1
  MISC_FEATURE (50)..(66): CDRH2
  MISC_FEATURE (99)..(106): CDRH3
QVQLQQSAAELARPGASVKMSCKASGYTFTDLSMHWIKQRPGQGLEWIGYITPSSGYTAYNQKFKGKTTLTADKSSSTAYMQLSSLTSEDSAVYYCARLILQRGAYWGQGTLVTVSAASTKGPSVFPLAPSSKSTSGGTAALGCLVKDYFPEPVTVSWNSGALTSGVHTFPAVLQSSGLYSLSSVVTVPSSSLGTQTYICNVNHKPSNTKVDKRVEPKSCDKTHTCPPCPAPELLGGPSVFLFPPKPKDTLMISRTPEVTCVVVDVSHEDPEVKFNWYVDGVEVHNAKTKPREEQYNSTYRVVSVLTVLHQDWLNGKEYKCKVSNKALPAPIEKTISKAKGQPREPQVYTLPPSREEMTKNQVSLTCLVKGFYPSDIAVEWESNGQPENNYKTTPPVLDSDGSFFLYSKLTVDKSRWQQGNVFSCSVMHEALHNHYTQKSLSLSPG

SEQ ID NO: 24 - protein, 218 aa, Artificial Sequence
  chimeric antibody with mouse variable domain and human constant domain
  DOMAIN (1)..(111): variable domain
  MISC_FEATURE (24)..(38): CDRL1
  MISC_FEATURE (54)..(60): CDRL2
  MISC_FEATURE (93)..(101): CDRL3
DIVLTQSPASLAVSLGQRATISCRASKNVDSYGNSFMHWYQQKPGQPPKLLIYRASNLESGIPARFGGSGSGTDFTLTINPVEADDVATYYCQQSNEDPLTFGAGTKLELKRTVAAPSVFIFPPSDEQLKSGTASVVCLLNNFYPREAKVQWKVDNALQSGNSQESVTEQDSKDSTYSLSSTLTLSKADYEKHKVYACEVTHQGLSSPVTKSFNRGEC

SEQ ID NO: 25 - protein, 446 aa, Artificial Sequence
  humanized antibody with mouse CDRs and human framework and constant regions
  DOMAIN (1)..(117): variable domain
  MISC_FEATURE (31)..(35): CDRH1
  MISC_FEATURE (50)..(66): CDRH2
  MISC_FEATURE (99)..(106): CDRH3
QVQLVQSGAEVKKPGSSVKVSCKASGYTFTDLSMHWIKQRPGQGLEWIGYITPSSGYTAYNQKFKGKTTLTADKSTSTAYMELSSLRSEDTAVYYCARLILQRGAYWGQGTLVTVSSASTKGPSVFPLAPSSKSTSGGTAALGCLVKDYFPEPVTVSWNSGALTSGVHTFPAVLQSSGLYSLSSVVTVPSSSLGTQTYICNVNHKPSNTKVDKRVEPKSCDKTHTCPPCPAPELLGGPSVFLFPPKPKDTLMISRTPEVTCVVVDVSHEDPEVKFNWYVDGVEVHNAKTKPREEQYNSTYRVVSVLTVLHQDWLNGKEYKCKVSNKALPAPIEKTISKAKGQPREPQVYTLPPSREEMTKNQVSLTCLVKGFYPSDIAVEWESNGQPENNYKTTPPVLDSDGSFFLYSKLTVDKSRWQQGNVFSCSVMHEALHNHYTQKSLSLSPG

SEQ ID NO: 26 - protein, 218 aa, Artificial Sequence
  humanized antibody with mouse CDRs and human framework and constant regions
  DOMAIN (1)..(111): variable domain
  MISC_FEATURE (24)..(38): CDRL1
  MISC_FEATURE (54)..(60): CDRL2
  MISC_FEATURE (93)..(101): CDRL3
DIVMTQSPDSLAVSLGERATINCRASKNVDSYGNSFMHWYQQKPGQPPKLLIYRASNLESGVPDRFSGSGSGTDFTLTISSLQAEDVAVYYCQQSNEDPLTFGQGTKLEIKRTVAAPSVFIFPPSDEQLKSGTASVVCLLNNFYPREAKVQWKVDNALQSGNSQESVTEQDSKDSTYSLSSTLTLSKADYEKHKVYACEVTHQGLSSPVTKSFNRGEC

SEQ ID NO: 27 - protein, 446 aa, Artificial Sequence; identical to SEQ ID NO: 25
  humanized antibody with mouse CDRs and human framework and constant regions
  DOMAIN (1)..(117): variable domain
  MISC_FEATURE (31)..(35): CDRH1
  MISC_FEATURE (50)..(66): CDRH2
  MISC_FEATURE (99)..(106): CDRH3

SEQ ID NO: 28 - protein, 218 aa, Artificial Sequence
  humanized antibody with mouse CDRs and human framework and constant regions
  DOMAIN (1)..(111): variable domain
  MISC_FEATURE (24)..(38): CDRL1
  MISC_FEATURE (54)..(60): CDRL2
  MISC_FEATURE (93)..(101): CDRL3
DIVLTQSPDSLAVSLGERATISCRASKNVDSYGNSFMHWYQQKPGQPPKLLIYRASNLESGVPDRFSGSGSGTDFTLTISSLQAEDVAVYYCQQSNEDPLTFGQGTKLEIKRTVAAPSVFIFPPSDEQLKSGTASVVCLLNNFYPREAKVQWKVDNALQSGNSQESVTEQDSKDSTYSLSSTLTLSKADYEKHKVYACEVTHQGLSSPVTKSFNRGEC

SEQ ID NO: 29 - protein, 446 aa, Artificial Sequence
  humanized antibody with mouse CDRs and human framework and constant regions
  DOMAIN (1)..(117): variable domain
  MISC_FEATURE (31)..(35): CDRH1
  MISC_FEATURE (50)..(66): CDRH2
  MISC_FEATURE (99)..(106): CDRH3
QVQLVQSGAEVKKPGSSVKVSCKASGYTFTDLSMHWVRQAPGQGLEWMGYITPSSGYTAYNQKFKGKTTLTADKSTSTAYMELSSLRSEDTAVYYCARLILQRGAYWGQGTLVTVSSASTKGPSVFPLAPSSKSTSGGTAALGCLVKDYFPEPVTVSWNSGALTSGVHTFPAVLQSSGLYSLSSVVTVPSSSLGTQTYICNVNHKPSNTKVDKRVEPKSCDKTHTCPPCPAPELLGGPSVFLFPPKPKDTLMISRTPEVTCVVVDVSHEDPEVKFNWYVDGVEVHNAKTKPREEQYNSTYRVVSVLTVLHQDWLNGKEYKCKVSNKALPAPIEKTISKAKGQPREPQVYTLPPSREEMTKNQVSLTCLVKGFYPSDIAVEWESNGQPENNYKTTPPVLDSDGSFFLYSKLTVDKSRWQQGNVFSCSVMHEALHNHYTQKSLSLSPG

SEQ ID NO: 30 - protein, 218 aa, Artificial Sequence
  humanized antibody with mouse CDRs and human framework and constant regions
  DOMAIN (1)..(111): variable domain
  MISC_FEATURE (24)..(38): CDRL1
  MISC_FEATURE (54)..(60): CDRL2
  MISC_FEATURE (93)..(101): CDRL3
DIVLTQSPDSLAVSLGERATINCRASKNVDSYGNSFMHWYQQKPGQPPKLLIYRASNLESGVPDRFSGSGSGTDFTLTISSLQAEDVAVYYCQQSNEDPLTFGQGTKLEIKRTVAAPSVFIFPPSDEQLKSGTASVVCLLNNFYPREAKVQWKVDNALQSGNSQESVTEQDSKDSTYSLSSTLTLSKADYEKHKVYACEVTHQGLSSPVTKSFNRGEC

SEQ ID NO: 31 - protein, 446 aa, Artificial Sequence
  humanized antibody with mouse CDRs and human framework and constant regions
  DOMAIN (1)..(117): variable domain
  MISC_FEATURE (31)..(35): CDRH1
  MISC_FEATURE (50)..(66): CDRH2
  MISC_FEATURE (99)..(106): CDRH3
QVQLVQSGAEVKKPGSSVKVSCKASGYTFTDLSMHWVRQAPGQGLEWMGYITPSSGYTAYNQKFKGKTTLTADKSTSTAYMELSSLRSEDTAVYYCARLILQRGAYWGQGTLVTVSSASTKGPSVFPLAPSSKSTSGGTAALGCLVKDYFPEPVTVSWNSGALTSGVHTFPAVLQSSGLYSLSSVVTVPSSSLGTQTYICNVNHKPSNTKVDKRVEPKSCDKTHTCPPCPAPELLGGPSVFLFPPKPKDTLMISRTPEVTCVVVDVEHEDPEVKFNWYVDGVEVHNAKTKPREEQYNSTYRVVSVLTVLHQDWLNGKEYKCKVSNKALPAPIEKTISKAKGQPREPQVYTLPPSREEMTKNQVSLTCLVKGFYPSDIAVEWESNGQPENNYKTTPPVLDSDGSFFLYSKLTVDKSRWQQGNVFSCSVMHEALHNHYTQKSLSLSPG

SEQ ID NO: 32 - protein, 446 aa, Artificial Sequence
  humanized antibody with mouse CDRs and human framework and constant regions
  DOMAIN (1)..(117): variable domain
  MISC_FEATURE (31)..(35): CDRH1
  MISC_FEATURE (50)..(66): CDRH2
  MISC_FEATURE (99)..(106): CDRH3
QVQLVQSGAEVKKPGSSVKVSCKASGYTFTDLSMHWVRQAPGQGLEWMGYITPSSGYTAYNQKFKGKTTLTADKSTSTAYMELSSLRSEDTAVYYCARLILQRGAYWGQGTLVTVSSASTKGPSVFPLAPSSKSTSGGTAALGCLVKDYFPEPVTVSWNSGALTSGVHTFPAVLQSSGLYSLSSVVTVPSSSLGTQTYICNVNHKPSNTKVDKRVEPKSCDKTHTCPPCPAPELLGGPSVFLFPPKPKDTLMISRTPEVTCVVVDVEHEDPEVKFNWYVDGVEVHNAKTKPREEQYNSTYRVVSVLTVLHQDWLNGKEYKCKVSNKAFPAPIEKTISKAKGQPREPQVYTLPPSREEMTKNQVSLTCLVKGFYPSDIAVEWESNGQPENNYKTTPPVLDSDGSFFLYSKLTVDKSRWQQGNVFSCSVMHEALHNHYTQKSLSLSPG

SEQ ID NO: 33 - protein, 446 aa, Artificial Sequence
  humanized antibody with mouse CDRs and human framework and constant regions
  DOMAIN (1)..(117): variable domain
  MISC_FEATURE (31)..(35): CDRH1
  MISC_FEATURE (50)..(66): CDRH2
  MISC_FEATURE (99)..(106): CDRH3
QVQLVQSGAEVKKPGSSVKVSCKASGYTFTDLSMHWVRQAPGQGLEWMGYITPSSGYTAYNQKFKGKTTLTADKSTSTAYMELSSLRSEDTAVYYCARLILQRGAYWGQGTLVTVSSASTKGPSVFPLAPSSKSTSGGTAALGCLVKDYFPEPVTVSWNSGALTSGVHTFPAVLQSSGLYSLSSVVTVPSSSLGTQTYICNVNHKPSNTKVDKRVEPKSCDKTHTCPPCPAPELLGGDSVFLFPPKPKDTLMISRTPEVTCVVVDVSHEDGEVKFNWYVDGVEVHNAKTKPREEQYNSTYRVVSVLTVLHQDWLNGKEYKCKVSNKALPAPIEKTISKAKGQPREPQVYTLPPSREEMTKNQVSLTCLVKGFYPSDIAVEWESNGQPENNYKTTPPVLDSDGSFFLYSKLTVDKSRWQQGNVFSCSVMHEALHNHYTQKSLSLSPG

SEQ ID NO: 34 - protein, 446 aa, Artificial Sequence
  humanized antibody with mouse CDRs and human framework and constant regions
QVQLVQSGAEVKKPGSSVKVSCKASGYTFTDLSMHWVRQAPGQGLEWMGYITPSSGYTAYNQKFKGKTTLTADKSTSTAYMELSSLRSEDTAVYYCARLILQRGAYWGQGTLVTVSSASTKGPSVFPLAPSSKSTSGGTAALGCLVKDYFPEPVTVSWNSGALTSGVHTFPAVLQSSGLYSLSSVVTVPSSSLGTQTYICNVNHKPSNTKVDKRVEPKSCDKTHTCPPCPAPELLGGDSVFLFPPKPKDTLMISRTPEVTCVVVDVSHEEGEVKFNWYVDGVEVHNAKTKPREEQYNSTYRVVSVLTVLHQDWLNGKEYKCKVSNKALPAPIEKTISKAKGQPREPQVYTLPPSREEMTKNQVSLTCLVKGFYPSDIAVEWESNGQPENNYKTTPPVLDSDGSFFLYSKLTVDKSRWQQGNVFSCSVMHEALHNHYTQKSLSLSPG

SEQ ID NO: 35 - protein, 446 aa, Artificial Sequence
  humanized antibody with mouse CDRs and human framework and constant regions
QVQLVQSGAEVKKPGSSVKVSCKASGYTFTDLSMHWVRQAPGQGLEWMGYITPSSGYTAYNQKFKGKTTLTADKSTSTAYMELSSLRSEDTAVYYCARLILQRGAYWGQGTLVTVSSASTKGPSVFPLAPSSKSTSGGTAALGCLVKDYFPEPVTVSWNSGALTSGVHTFPAVLQSSGLYSLSSVVTVPSSSLGTQTYICNVNHKPSNTKVDKRVEPKSCDKTHTCPPCPAPELLGDDSVFLFPPKPKDTLMISRTPEVTCVVVDVSDEDGEVKFNWYVDGVEVHNAKTKPREEQYNSTYRVVSVLTVLHQDWLNGKEYKCKVSNKALPAPIEKTISKAKGQPREPQVYTLPPSREEMTKNQVSLTCLVKGFYPSDIAVEWESNGQPENNYKTTPPVLDSDGSFFLYSKLTVDKSRWQQGNVFSCSVMHEALHNHYTQKSLSLSPG

SEQ ID NO: 36 - protein, 446 aa, Artificial Sequence
  humanized antibody with mouse CDRs and human framework and constant regions
  DOMAIN (1)..(117): variable domain
  MISC_FEATURE (31)..(35): CDRH1
  MISC_FEATURE (50)..(66): CDRH2
  MISC_FEATURE (99)..(106): CDRH3
QVQLVQSGAEVKKPGSSVKVSCKASGYTFTDLSMHWVRQAPGQGLEWMGYITPSSGYTAYNQKFKGKTTLTADKSTSTAYMELSSLRSEDTAVYYCARLILQRGAYWGQGTLVTVSSASTKGPSVFPLAPSSKSTSGGTAALGCLVKDYFPEPVTVSWNSGALTSGVHTFPAVLQSSGLYSLSSVVTVPSSSLGTQTYICNVNHKPSNTKVDKRVEPKSCDKTHTCPPCPAPELLGDDSVFLFPPKPKDTLMISRTPEVTCVVVDVSHEDGEVKFNWYVDGVEVHNAKTKPREEQYNSTYRVVSVLTVLHQDWLNGKEYKCKVSNKALPRPIEKTISKAKGQPREPQVYTLPPSREEMTKNQVSLTCLVKGFYPSDIAVEWESNGQPENNYKTTPPVLDSDGSFFLYSKLTVDKSRWQQGNVFSCSVMHEALHNHYTQKSLSLSPG

SEQ ID NO: 37 - protein, 446 aa, Artificial Sequence
  humanized antibody with mouse CDRs and human framework and constant regions
QVQLVQSGAEVKKPGSSVKVSCKASGYTFTDLSMHWVRQAPGQGLEWMGYITPSSGYTAYNQKFKGKTTLTADKSTSTAYMELSSLRSEDTAVYYCARLILQRGAYWGQGTLVTVSSASTKGPSVFPLAPSSKSTSGGTAALGCLVKDYFPEPVTVSWNSGALTSGVHTFPAVLQSSGLYSLSSVVTVPSSSLGTQTYICNVNHKPSNTKVDKRVEPKSCDKTHTCPPCPAPELLGDDSVFLFPPKPKDTLMISRTPEVTCVVVDVSHEEGEVKFNWYVDGVEVHNAKTKPREEQYNSTYRVVSVLTVLHQDWLNGKEYKCKVSNKALPRPIEKTISKAKGQPREPQVYTLPPSREEMTKNQVSLTCLVKGFYPSDIAVEWESNGQPENNYKTTPPVLDSDGSFFLYSKLTVDKSRWQQGNVFSCSVMHEALHNHYTQKSLSLSPG

SEQ ID NO: 38 - protein, 446 aa, Artificial Sequence
  humanized antibody with mouse CDRs and human framework and constant regions
  DOMAIN (1)..(117): variable domain
  MISC_FEATURE (31)..(35): CDRH1
  MISC_FEATURE (50)..(66): CDRH2
  MISC_FEATURE (99)..(106): CDRH3
QVQLVQSGAEVKKPGSSVKVSCKASGYTFTDLSMHWVRQAPGQGLEWMGYITPSSGYTAYNQKFKGKTTLTADKSTSTAYMELSSLRSEDTAVYYCARLILQRGAYWGQGTLVTVSSASTKGPSVFPLAPSSKSTSGGTAALGCLVKDYFPEPVTVSWNSGALTSGVHTFPAVLQSSGLYSLSSVVTVPSSSLGTQTYICNVNHKPSNTKVDKRVEPKSCDKTHTCPPCPAPELLGDDSVFLFPPKPKDTLMISRTPEVTCVVVDVSDEDGEVKFNWYVDGVEVHNAKTKPREEQYNSTYRVVSVLTVLHQDWLNGKEYKCKVSNKALPRPIEKTISKAKGQPREPQVYTLPPSREEMTKNQVSLTCLVKGFYPSDIAVEWESNGQPENNYKTTPPVLDSDGSFFLYSKLTVDKSRWQQGNVFSCSVMHEALHNHYTQKSLSLSPG

SEQ ID NO: 39 - protein, 446 aa, Artificial Sequence
  humanized antibody with mouse CDRs and human framework and constant regions
  DOMAIN (1)..(117): variable domain
  MISC_FEATURE (31)..(35): CDRH1
  MISC_FEATURE (50)..(66): CDRH2
  MISC_FEATURE (99)..(106): CDRH3
QVQLVQSGAEVKKPGSSVKVSCKASGYTFTDLSMHWVRQAPGQGLEWMGYITPSSGYTAYNQKFKGKTTLTADKSTSTAYMELSSLRSEDTAVYYCARLILQRGAYWGQGTLVTVSSASTKGPSVFPLAPSSKSTSGGTAALGCLVKDYFPEPVTVSWNSGALTSGVHTFPAVLQSSGLYSLSSVVTVPSSSLGTQTYICNVNHKPSNTKVDKRVEPKSCDKTHTCPPCPAPDLLGDDSVFLFPPKPKDTLMISRTPEVTCVVVDVSDEDGEVKFNWYVDGVEVHNAKTKPREEQYNSTYRVVSVLTVLHQDWLNGKEYKCKVSNKALPRPIEKTISKAKGQPREPQVYTLPPSREEMTKNQVSLTCLVKGFYPSDIAVEWESNGQPENNYKTTPPVLDSDGSFFLYSKLTVDKSRWQQGNVFSCSVMHEALHNHYTQKSLSLSPG

SEQ ID NO: 40 - protein, 451 aa, Artificial Sequence
  chimeric antibody with mouse variable domain and human constant domain
  DOMAIN (1)..(122): variable domain
  MISC_FEATURE (31)..(35): CDRH1
  MISC_FEATURE (50)..(66): CDRH2
  MISC_FEATURE (99)..(111): CDRH3
QVQFQQSGAELARPGASVKLSCKASGYTFTSYWMQWVKQRPGQGLEWIGTIYPGDGDSRYNQKFKGKALLTADKSSSIAYMQLNSLASEDSAVYFCARFSLYDGYPYYFDYWGQGTTLTVSSASTKGPSVFPLAPSSKSTSGGTAALGCLVKDYFPEPVTVSWNSGALTSGVHTFPAVLQSSGLYSLSSVVTVPSSSLGTQTYICNVNHKPSNTKVDKRVEPKSCDKTHTCPPCPAPELLGGPSVFLFPPKPKDTLMISRTPEVTCVVVDVSHEDPEVKFNWYVDGVEVHNAKTKPREEQYNSTYRVVSVLTVLHQDWLNGKEYKCKVSNKALPAPIEKTISKAKGQPREPQVYTLPPSREEMTKNQVSLTCLVKGFYPSDIAVEWESNGQPENNYKTTPPVLDSDGSFFLYSKLTVDKSRWQQGNVFSCSVMHEALHNHYTQKSLSLSPG

SEQ ID NO: 41 - protein, 219 aa, Artificial Sequence
  chimeric antibody with mouse variable domain and human constant domain
  DOMAIN (1)..(112): variable domain
  MISC_FEATURE (24)..(39): CDRL1
  MISC_FEATURE (55)..(61): CDRL2
  MISC_FEATURE (94)..(102): CDRL3
DVVMTQTPLSLPVSLGDQASISCRSSQSLVHRNGNTYLHWYLQKPGQSPKLLIYRVSNRFSGVPDRFSGSGSGTDFTLKISRVEAEDLGIYFCSQSTHFPYTFGGGTKLEIKRTVAAPSVFIFPPSDEQLKSGTASVVCLLNNFYPREAKVQWKVDNALQSGNSQESVTEQDSKDSTYSLSSTLTLSKADYEKHKVYACEVTHQGLSSPVTKSFNRGEC

SEQ ID NO: 42 - protein, 451 aa, Artificial Sequence
  humanized antibody with mouse CDRs and human framework and constant regions
  DOMAIN (1)..(122): variable domain
  MISC_FEATURE (31)..(35): CDRH1
  MISC_FEATURE (50)..(66): CDRH2
  MISC_FEATURE (99)..(111): CDRH3
QVQFVQSGAEVKKPGSSVKVSCKASGYTFTSYWMQWVRQAPGQGLEWMGTIYPGDGDSRYNQKFKGKALLTADKSTSTAYMELSSLRSEDTAVYYCARFSLYDGYPYYFDYWGQGTTVTVSSASTKGPSVFPLAPSSKSTSGGTAALGCLVKDYFPEPVTVSWNSGALTSGVHTFPAVLQSSGLYSLSSVVTVPSSSLGTQTYICNVNHKPSNTKVDKRVEPKSCDKTHTCPPCPAPELLGGPSVFLFPPKPKDTLMISRTPEVTCVVVDVSHEDPEVKFNWYVDGVEVHNAKTKPREEQYNSTYRVVSVLTVLHQDWLNGKEYKCKVSNKALPAPIEKTISKAKGQPREPQVYTLPPSREEMTKNQVSLTCLVKGFYPSDIAVEWESNGQPENNYKTTPPVLDSDGSFFLYSKLTVDKSRWQQGNVFSCSVMHEALHNHYTQKSLSLSPG

SEQ ID NO: 43 - protein, 219 aa, Artificial Sequence
  humanized antibody with mouse CDRs and human framework and constant regions
  DOMAIN (1)..(112): variable domain
  MISC_FEATURE (24)..(39): CDRL1
  MISC_FEATURE (55)..(61): CDRL2
  MISC_FEATURE (94)..(102): CDRL3
DIVMTQSPLSLPVTPGEPASISCRSSQSLVHRNGNTYLHWYLQKPGQSPQLLIYRVSNRFSGVPDRFSGSGSGTDFTLKISRVEAEDVGVYYCSQSTHFPYTFGGGTKVEIKRTVAAPSVFIFPPSDEQLKSGTASVVCLLNNFYPREAKVQWKVDNALQSGNSQESVTEQDSKDSTYSLSSTLTLSKADYEKHKVYACEVTHQGLSSPVTKSFNRGEC

SEQ ID NO: 44 - protein, 451 aa, Artificial Sequence
  humanized antibody with mouse CDRs and human framework and constant regions
  DOMAIN (1)..(122): variable domain
  MISC_FEATURE (31)..(35): CDRH1
  MISC_FEATURE (50)..(66): CDRH2
  MISC_FEATURE (99)..(111): CDRH3
QVQFVQSGAEVKKPGSSVKVSCKASGYTFTSYWMQWVRQAPGQGLEWMGTIYPGDGDSRYNQKFKGKALLTADKSTSTAYMELSSLRSEDTAVYYCARFSLYEGYPYYFDYWGQGTTVTVSSASTKGPSVFPLAPSSKSTSGGTAALGCLVKDYFPEPVTVSWNSGALTSGVHTFPAVLQSSGLYSLSSVVTVPSSSLGTQTYICNVNHKPSNTKVDKRVEPKSCDKTHTCPPCPAPELLGGPSVFLFPPKPKDTLMISRTPEVTCVVVDVSHEDPEVKFNWYVDGVEVHNAKTKPREEQYNSTYRVVSVLTVLHQDWLNGKEYKCKVSNKALPAPIEKTISKAKGQPREPQVYTLPPSREEMTKNQVSLTCLVKGFYPSDIAVEWESNGQPENNYKTTPPVLDSDGSFFLYSKLTVDKSRWQQGNVFSCSVMHEALHNHYTQKSLSLSPG

SEQ ID NO: 45 - protein, 219 aa, Artificial Sequence; identical to SEQ ID NO: 43
  humanized antibody with mouse CDRs and human framework and constant regions
  DOMAIN (1)..(112): variable domain
  MISC_FEATURE (24)..(39): CDRL1
  MISC_FEATURE (55)..(61): CDRL2
  MISC_FEATURE (94)..(102): CDRL3

SEQ ID NO: 46 - protein, 451 aa, Artificial Sequence; identical to SEQ ID NO: 44
  humanized antibody with mouse CDRs and human framework and constant regions
  DOMAIN (1)..(122): variable domain
  MISC_FEATURE (31)..(35): CDRH1
  MISC_FEATURE (50)..(66): CDRH2
  MISC_FEATURE (99)..(111): CDRH3

SEQ ID NO: 47 - protein, 219 aa, Artificial Sequence
  humanized antibody with mouse CDRs and human framework and constant regions
  DOMAIN (1)..(112): variable domain
  MISC_FEATURE (24)..(39): CDRL1
  MISC_FEATURE (55)..(61): CDRL2
  MISC_FEATURE (94)..(102): CDRL3
DIVMTQSPLSLPVTPGEPASISCRSSQSLVHRNANTYLHWYLQKPGQSPQLLIYRVSNRFSGVPDRFSGSGSGTDFTLKISRVEAEDVGVYYCSQSTHFPYTFGGGTKVEIKRTVAAPSVFIFPPSDEQLKSGTASVVCLLNNFYPREAKVQWKVDNALQSGNSQESVTEQDSKDSTYSLSSTLTLSKADYEKHKVYACEVTHQGLSSPVTKSFNRGEC

SEQ ID NO: 48 - protein, 451 aa, Artificial Sequence
  humanized antibody with mouse CDRs and human framework and constant regions
  DOMAIN (1)..(122): variable domain
  MISC_FEATURE (31)..(35): CDRH1
  MISC_FEATURE (50)..(66): CDRH2
  MISC_FEATURE (99)..(111): CDRH3
QVQFVQSGAEVKKPGSSVKVSCKASGYTFTSYWMQWVRQAPGQGLEWMGTIYPGDSDSRYNQKFKGKALLTADKSTSTAYMELSSLRSEDTAVYYCARFSLYEGYPYYFDYWGQGTTVTVSSASTKGPSVFPLAPSSKSTSGGTAALGCLVKDYFPEPVTVSWNSGALTSGVHTFPAVLQSSGLYSLSSVVTVPSSSLGTQTYICNVNHKPSNTKVDKRVEPKSCDKTHTCPPCPAPELLGGPSVFLFPPKPKDTLMISRTPEVTCVVVDVSHEDPEVKFNWYVDGVEVHNAKTKPREEQYNSTYRVVSVLTVLHQDWLNGKEYKCKVSNKALPAPIEKTISKAKGQPREPQVYTLPPSREEMTKNQVSLTCLVKGFYPSDIAVEWESNGQPENNYKTTPPVLDSDGSFFLYSKLTVDKSRWQQGNVFSCSVMHEALHNHYTQKSLSLSPG

SEQ ID NO: 49 - protein, 219 aa, Artificial Sequence; identical to SEQ ID NO: 43
  humanized antibody with mouse CDRs and human framework and constant regions
  DOMAIN (1)..(112): variable domain
  MISC_FEATURE (24)..(39): CDRL1
  MISC_FEATURE (55)..(61): CDRL2
  MISC_FEATURE (94)..(102): CDRL3

SEQ ID NO: 50 - protein, 451 aa, Artificial Sequence; identical to SEQ ID NO: 48
  humanized antibody with mouse CDRs and human framework and constant regions
  DOMAIN (1)..(122): variable domain
  MISC_FEATURE (31)..(35): CDRH1
  MISC_FEATURE (50)..(66): CDRH2
  MISC_FEATURE (99)..(111): CDRH3

SEQ ID NO: 51 - protein, 219 aa, Artificial Sequence; identical to SEQ ID NO: 47
  humanized antibody with mouse CDRs and human framework and constant regions
  DOMAIN (1)..(112): variable domain
  MISC_FEATURE (24)..(39): CDRL1
  MISC_FEATURE (55)..(61): CDRL2
  MISC_FEATURE (94)..(102): CDRL3

SEQ ID NO: 52 - protein, 442 aa, Artificial Sequence
  chimeric antibody with mouse variable domain and human constant domain
  DOMAIN (1)..(113): variable domain
  MISC_FEATURE (31)..(35): CDRH1
  MISC_FEATURE (50)..(66): CDRH2
  MISC_FEATURE (99)..(102): CDRH3
EVLLQQSGPELVKPGASVKIPCKASGYKFTDYNMDWVKQSHGKSLEWIGDINPKNGGTIYNLKFKGKATLTVDMSSSTAYMELRSLTSEDTAVYYCVRRMDYWGQGTSVTVSSASTKGPSVFPLAPSSKSTSGGTAALGCLVKDYFPEPVTVSWNSGALTSGVHTFPAVLQSSGLYSLSSVVTVPSSSLGTQTYICNVNHKPSNTKVDKRVEPKSCDKTHTCPPCPAPELLGGPSVFLFPPKPKDTLMISRTPEVTCVVVDVSHEDPEVKFNWYVDGVEVHNAKTKPREEQYNSTYRVVSVLTVLHQDWLNGKEYKCKVSNKALPAPIEKTISKAKGQPREPQVYTLPPSREEMTKNQVSLTCLVKGFYPSDIAVEWESNGQPENNYKTTPPVLDSDGSFFLYSKLTVDKSRWQQGNVFSCSVMHEALHNHYTQKSLSLSPG

SEQ ID NO: 53 - protein, 214 aa, Artificial Sequence
  chimeric antibody with mouse variable domain and human constant domain
  DOMAIN (1)..(107): variable domain
  MISC_FEATURE (24)..(34): CDRL1
  MISC_FEATURE (50)..(56): CDRL2
  MISC_FEATURE (89)..(97): CDRL3
DIQMTQTTSSLSASLGDRVTISCRASQDISNYLNWYQQKPDGTVKLLIYYISRLHSGVPSRFRGSGSGTDFSLTISNLEQEDIATYFCQQGNTLPYTFGGGTNLEIKRTVAAPSVFIFPPSDEQLKSGTASVVCLLNNFYPREAKVQWKVDNALQSGNSQESVTEQDSKDSTYSLSSTLTLSKADYEKHKVYACEVTHQGLSSPVTKSFNRGEC

SEQ ID NO: 54 - protein, 442 aa, Artificial Sequence
  humanized antibody with mouse CDRs and human framework and constant regions
  DOMAIN (1)..(113): variable domain
  MISC_FEATURE (31)..(35): CDRH1
  MISC_FEATURE (50)..(66): CDRH2
  MISC_FEATURE (99)..(102): CDRH3
QVQLVQSGAEVKKPGASVKVSCKASGYTFTDYNMDWVRQAPGQGLEWMGDINPKNGGTIYNLKFKGRVTLTTDTSTSTAYMELRSLRSDDTAVYYCVRRMDYWGQGTTVTVSSASTKGPSVFPLAPSSKSTSGGTAALGCLVKDYFPEPVTVSWNSGALTSGVHTFPAVLQSSGLYSLSSVVTVPSSSLGTQTYICNVNHKPSNTKVDKRVEPKSCDKTHTCPPCPAPELLGGPSVFLFPPKPKDTLMISRTPEVTCVVVDVSHEDPEVKFNWYVDGVEVHNAKTKPREEQYNSTYRVVSVLTVLHQDWLNGKEYKCKVSNKALPAPIEKTISKAKGQPREPQVYTLPPSREEMTKNQVSLTCLVKGFYPSDIAVEWESNGQPENNYKTTPPVLDSDGSFFLYSKLTVDKSRWQQGNVFSCSVMHEALHNHYTQKSLSLSPG

SEQ ID NO: 55 - protein, 214 aa, Artificial Sequence
  humanized antibody with mouse CDRs and human framework and constant regions
  DOMAIN (1)..(107): variable domain
  MISC_FEATURE (24)..(34): CDRL1
  MISC_FEATURE (50)..(56): CDRL2
  MISC_FEATURE (89)..(97): CDRL3
DIQMTQSPSSLSASVGDRVTITCRASQDISNYLNWYQQKPGKVPKLLIYYISRLHSGVPSRFSGSGSGTDFTLTISSLQPEDVATYYCQQGNTLPYTFGGGTKVEIKRTVAAPSVFIFPPSDEQLKSGTASVVCLLNNFYPREAKVQWKVDNALQSGNSQESVTEQDSKDSTYSLSSTLTLSKADYEKHKVYACEVTHQGLSSPVTKSFNRGEC

SEQ ID NO: 56 - protein, 442 aa, Artificial Sequence
  humanized antibody with mouse CDRs and human framework and constant regions
  DOMAIN (1)..(113): variable domain
  MISC_FEATURE (31)..(35): CDRH1
  MISC_FEATURE (50)..(66): CDRH2
  MISC_FEATURE (99)..(102): CDRH3
QVQLVQSGAEVKKPGASVKVSCKASGYTFTDYNMDWVRQAPGQGLEWMGDINPKNAGTIYNLKFKGRVTLTVDTSTSTAYMELRSLRSDDTAVYYCVRRMDYWGQGTTVTVSSASTKGPSVFPLAPSSKSTSGGTAALGCLVKDYFPEPVTVSWNSGALTSGVHTFPAVLQSSGLYSLSSVVTVPSSSLGTQTYICNVNHKPSNTKVDKRVEPKSCDKTHTCPPCPAPELLGGPSVFLFPPKPKDTLMISRTPEVTCVVVDVSHEDPEVKFNWYVDGVEVHNAKTKPREEQYNSTYRVVSVLTVLHQDWLNGKEYKCKVSNKALPAPIEKTISKAKGQPREPQVYTLPPSREEMTKNQVSLTCLVKGFYPSDIAVEWESNGQPENNYKTTPPVLDSDGSFFLYSKLTVDKSRWQQGNVFSCSVMHEALHNHYTQKSLSLSPG

SEQ ID NO: 57 - protein, 214 aa, Artificial Sequence; identical to SEQ ID NO: 55
  humanized antibody with mouse CDRs and human framework and constant regions
  DOMAIN (1)..(107): variable domain
  MISC_FEATURE (24)..(34): CDRL1
  MISC_FEATURE (50)..(56): CDRL2
  MISC_FEATURE (89)..(97): CDRL3

SEQ ID NO: 58 - protein, 441 aa, Artificial Sequence
  chimeric antibody with mouse variable domain and human constant domain
  DOMAIN (1)..(112): variable domain
  MISC_FEATURE (31)..(35): CDRH1
  MISC_FEATURE (50)..(66): CDRH2
  MISC_FEATURE (99)..(101): CDRH3
EVQLVESGGGLVKPGGSLKLSCAASGFTFSSYAMSWVRQSPEKRLEWVAEISGGGSYTYYPDTVTGRFTISRDNAKNTLYLEMSSLRSEDTAMYYCASRAYWGQGTLVTVSAASTKGPSVFPLAPSSKSTSGGTAALGCLVKDYFPEPVTVSWNSGALTSGVHTFPAVLQSSGLYSLSSVVTVPSSSLGTQTYICNVNHKPSNTKVDKRVEPKSCDKTHTCPPCPAPELLGGPSVFLFPPKPKDTLMISRTPEVTCVVVDVSHEDPEVKFNWYVDGVEVHNAKTKPREEQYNSTYRVVSVLTVLHQDWLNGKEYKCKVSNKALPAPIEKTISKAKGQPREPQVYTLPPSREEMTKNQVSLTCLVKGFYPSDIAVEWESNGQPENNYKTTPPVLDSDGSFFLYSKLTVDKSRWQQGNVFSCSVMHEALHNHYTQKSLSLSPG

SEQ ID NO: 59 - protein, 219 aa, Artificial Sequence
  chimeric antibody with mouse variable domain and human constant domain
  DOMAIN (1)..(112): variable domain
  MISC_FEATURE (24)..(39): CDRL1
  MISC_FEATURE (55)..(61): CDRL2
  MISC_FEATURE (94)..(102): CDRL3
DVLMTQTPLSLPVSLGDQASISCRSSQSIVHSNGNTYFEWYLQKPGQSPKLLIYKVSNRFSGVPDRFSGSGSGTDFTLKISRVEAEDLGVYYCFQGSHVPYTFGGGTKLEIKRTVAAPSVFIFPPSDEQLKSGTASVVCLLNNFYPREAKVQWKVDNALQSGNSQESVTEQDSKDSTYSLSSTLTLSKADYEKHKVYACEVTHQGLSSPVTKSFNRGEC

SEQ ID NO: 60 - protein, 441 aa, Artificial Sequence
  humanized antibody with mouse CDRs and human framework and constant regions
  DOMAIN (1)..(112): variable domain
  MISC_FEATURE (31)..(35): CDRH1
  MISC_FEATURE (50)..(66): CDRH2
  MISC_FEATURE (99)..(101): CDRH3
EVQLVESGGGLVKPGGSLRLSCAASGFTFSSYAMSWVRQAPGKGLEWVSEISGGGSYTYYPDTVTGRFTISRDNAKNSLYLQMNSLRAEDTAVYYCASRAYWGQGTLVTVSSASTKGPSVFPLAPSSKSTSGGTAALGCLVKDYFPEPVTVSWNSGALTSGVHTFPAVLQSSGLYSLSSVVTVPSSSLGTQTYICNVNHKPSNTKVDKRVEPKSCDKTHTCPPCPAPELLGGPSVFLFPPKPKDTLMISRTPEVTCVVVDVSHEDPEVKFNWYVDGVEVHNAKTKPREEQYNSTYRVVSVLTVLHQDWLNGKEYKCKVSNKALPAPIEKTISKAKGQPREPQVYTLPPSREEMTKNQVSLTCLVKGFYPSDIAVEWESNGQPENNYKTTPPVLDSDGSFFLYSKLTVDKSRWQQGNVFSCSVMHEALHNHYTQKSLSLSPG

SEQ ID NO: 61 - protein, 441 aa, Artificial Sequence
  humanized antibody with mouse CDRs and human framework and constant regions
  DOMAIN (1)..(112): variable domain
  MISC_FEATURE (31)..(35): CDRH1
  MISC_FEATURE (50)..(66): CDRH2
  MISC_FEATURE (99)..(101): CDRH3
EVQLVESGGGLVKPGGSLRLSCAASGFTFSSYAMSWVRQAPGKGLEWVSEISGGGSYTYYPDTVTGRFTISRDNAKNSLYLQMNSLRAEDTAVYYCASRAYWGQGTLVTVSSASTKGPSVFPLAPSSKSTSGGTAALGCLVKDYFPEPVTVSWNSGALTSGVHTFPAVLQSSGLYSLSSVVTVPSSSLGTQTYICNVNHKPSNTKVDKRVEPKSCDKTHTCPPCPAPELLGDDSVFLFPPKPKDTLMISRTPEVTCVVVDVSHEDGEVKFNWYVDGVEVHNAKTKPREEQYNSTYRVVSVLTVLHQDWLNGKEYKCKVSNKALPRPIEKTISKAKGQPREPQVYTLPPSREEMTKNQVSLTCLVKGFYPSDIAVEWESNGQPENNYKTTPPVLDSDGSFFLYSKLTVDKSRWQQGNVFSCSVMHEALHNHYTQKSLSLSPG

SEQ ID NO: 62 - protein, 219 aa, Artificial Sequence
  humanized antibody with mouse CDRs and human framework and constant regions
  DOMAIN (1)..(112): variable domain
  MISC_FEATURE (24)..(39): CDRL1
  MISC_FEATURE (55)..(61): CDRL2
  MISC_FEATURE (94)..(102): CDRL3
DIVMTQTPLSLPVTPGEPASISCRSSQSIVHSNGNTYFEWYLQKPGQSPQLLIYKVSNRFSGVPDRFSGSGSGTDFTLKISRVEAEDVGVYYCFQGSHVPYTFGGGTKVEIKRTVAAPSVFIFPPSDEQLKSGTASVVCLLNNFYPREAKVQWKVDNALQSGNSQESVTEQDSKDSTYSLSSTLTLSKADYEKHKVYACEVTHQGLSSPVTKSFNRGEC

SEQ ID NO: 63 - protein, 441 aa, Artificial Sequence; identical to SEQ ID NO: 60
  humanized antibody with mouse CDRs and human framework and constant regions
  DOMAIN (1)..(112): variable domain
  MISC_FEATURE (31)..(35): CDRH1
  MISC_FEATURE (50)..(66): CDRH2
  MISC_FEATURE (99)..(101): CDRH3

SEQ ID NO: 64 - protein, 219 aa, Artificial Sequence
  humanized antibody with mouse CDRs and human framework and constant regions
  DOMAIN (1)..(112): variable domain
  MISC_FEATURE (24)..(39): CDRL1
  MISC_FEATURE (55)..(61): CDRL2
  MISC_FEATURE (94)..(102): CDRL3
DIVMTQTPLSLPVTPGEPASISCRSSQSIVHSQGNTYFEWYLQKPGQSPQLLIYKVSNRFSGVPDRFSGSGSGTDFTLKISRVEAEDVGVYYCFQGSHVPYTFGGGTKVEIKRTVAAPSVFIFPPSDEQLKSGTASVVCLLNNFYPREAKVQWKVDNALQSGNSQESVTEQDSKDSTYSLSSTLTLSKADYEKHKVYACEVTHQGLSSPVTKSFNRGEC

SEQ ID NO: 65 - protein, 329 aa, Homo sapiens
ASTKGPSVFPLAPSSKSTSGGTAALGCLVKDYFPEPVTVSWNSGALTSGVHTFPAVLQSSGLYSLSSVVTVPSSSLGTQTYICNVNHKPSNTKVDKRVEPKSCDKTHTCPPCPAPELLGGPSVFLFPPKPKDTLMISRTPEVTCVVVDVSHEDPEVKFNWYVDGVEVHNAKTKPREEQYNSTYRVVSVLTVLHQDWLNGKEYKCKVSNKALPAPIEKTISKAKGQPREPQVYTLPPSREEMTKNQVSLTCLVKGFYPSDIAVEWESNGQPENNYKTTPPVLDSDGSFFLYSKLTVDKSRWQQGNVFSCSVMHEALHNHYTQKSLSLSPG

SEQ ID NO: 66 - protein, 329 aa, Artificial Sequence
  variant of human IgG1f constant domain
ASTKGPSVFPLAPSSKSTSGGTAALGCLVKDYFPEPVTVSWNSGALTSGVHTFPAVLQSSGLYSLSSVVTVPSSSLGTQTYICNVNHKPSNTKVDKRVEPKSCDKTHTCPPCPAPELLGGPSVFLFPPKPKDTLMISRTPEVTCVVVDVEHEDPEVKFNWYVDGVEVHNAKTKPREEQYNSTYRVVSVLTVLHQDWLNGKEYKCKVSNKALPAPIEKTISKAKGQPREPQVYTLPPSREEMTKNQVSLTCLVKGFYPSDIAVEWESNGQPENNYKTTPPVLDSDGSFFLYSKLTVDKSRWQQGNVFSCSVMHEALHNHYTQKSLSLSPG

SEQ ID NO: 67 - protein, 329 aa, Artificial Sequence
  variant of human IgG1f constant domain
ASTKGPSVFPLAPSSKSTSGGTAALGCLVKDYFPEPVTVSWNSGALTSGVHTFPAVLQSSGLYSLSSVVTVPSSSLGTQTYICNVNHKPSNTKVDKRVEPKSCDKTHTCPPCPAPELLGGPSVFLFPPKPKDTLMISRTPEVTCVVVDVEHEDPEVKFNWYVDGVEVHNAKTKPREEQYNSTYRVVSVLTVLHQDWLNGKEYKCKVSNKAFPAPIEKTISKAKGQPREPQVYTLPPSREEMTKNQVSLTCLVKGFYPSDIAVEWESNGQPENNYKTTPPVLDSDGSFFLYSKLTVDKSRWQQGNVFSCSVMHEALHNHYTQKSLSLSPG

SEQ ID NO: 68 - protein, 329 aa, Artificial Sequence
  variant of human IgG1f constant domain
ASTKGPSVFPLAPSSKSTSGGTAALGCLVKDYFPEPVTVSWNSGALTSGVHTFPAVLQSSGLYSLSSVVTVPSSSLGTQTYICNVNHKPSNTKVDKRVEPKSCDKTHTCPPCPAPELLGGDSVFLFPPKPKDTLMISRTPEVTCVVVDVSHEDPEVKFNWYVDGVEVHNAKTKPREEQYNSTYRVVSVLTVLHQDWLNGKEYKCKVSNKALPAPIEKTISKAKGQPREPQVYTLPPSREEMTKNQVSLTCLVKGFYPSDIAVEWESNGQPENNYKTTPPVLDSDGSFFLYSKLTVDKSRWQQGNVFSCSVMHEALHNHYTQKSLSLSPG

SEQ ID NO: 69 - protein, 329 aa, Artificial Sequence
  variant of human IgG1f constant domain
ASTKGPSVFPLAPSSKSTSGGTAALGCLVKDYFPEPVTVSWNSGALTSGVHTFPAVLQSSGLYSLSSVVTVPSSSLGTQTYICNVNHKPSNTKVDKRVEPKSCDKTHTCPPCPAPELLGGDSVFLFPPKPKDTLMISRTPEVTCVVVDVSHEDGEVKFNWYVDGVEVHNAKTKPREEQYNSTYRVVSVLTVLHQDWLNGKEYKCKVSNKALPAPIEKTISKAKGQPREPQVYTLPPSREEMTKNQVSLTCLVKGFYPSDIAVEWESNGQPENNYKTTPPVLDSDGSFFLYSKLTVDKSRWQQGNVFSCSVMHEALHNHYTQKSLSLSPG

SEQ ID NO: 70 - protein, 329 aa, Artificial Sequence
  variant of human IgG1f constant domain
ASTKGPSVFPLAPSSKSTSGGTAALGCLVKDYFPEPVTVSWNSGALTSGVHTFPAVLQSSGLYSLSSVVTVPSSSLGTQTYICNVNHKPSNTKVDKRVEPKSCDKTHTCPPCPAPELLGGDSVFLFPPKPKDTLMISRTPEVTCVVVDVSHEEGEVKFNWYVDGVEVHNAKTKPREEQYNSTYRVVSVLTVLHQDWLNGKEYKCKVSNKALPAPIEKTISKAKGQPREPQVYTLPPSREEMTKNQVSLTCLVKGFYPSDIAVEWESNGQPENNYKTTPPVLDSDGSFFLYSKLTVDKSRWQQGNVFSCSVMHEALHNHYTQKSLSLSPG

SEQ ID NO: 71 - protein, 329 aa, Artificial Sequence
  variant of human IgG1f constant domain
ASTKGPSVFPLAPSSKSTSGGTAALGCLVKDYFPEPVTVSWNSGALTSGVHTFPAVLQSSGLYSLSSVVTVPSSSLGTQTYICNVNHKPSNTKVDKRVEPKSCDKTHTCPPCPAPDLLGGDSVFLFPPKPKDTLMISRTPEVTCVVVDVSHEDGEVKFNWYVDGVEVHNAKTKPREEQYNSTYRVVSVLTVLHQDWLNGKEYKCKVSNKALPRPIEKTISKAKGQPREPQVYTLPPSREEMTKNQVSLTCLVKGFYPSDIAVEWESNGQPENNYKTTPPVLDSDGSFFLYSKLTVDKSRWQQGNVFSCSVMHEALHNHYTQKSLSLSPG

SEQ ID NO: 72 - protein, 329 aa, Artificial Sequence
  variant of human IgG1f constant domain
ASTKGPSVFPLAPSSKSTSGGTAALGCLVKDYFPEPVTVSWNSGALTSGVHTFPAVLQSSGLYSLSSVVTVPSSSLGTQTYICNVNHKPSNTKVDKRVEPKSCDKTHTCPPCPAPELLGDDSVFLFPPKPKDTLMISRTPEVTCVVVDVSDEDGEVKFNWYVDGVEVHNAKTKPREEQYNSTYRVVSVLTVLHQDWLNGKEYKCKVSNKALPAPIEKTISKAKGQPREPQVYTLPPSREEMTKNQVSLTCLVKGFYPSDIAVEWESNGQPENNYKTTPPVLDSDGSFFLYSKLTVDKSRWQQGNVFSCSVMHEALHNHYTQKSLSLSPG

SEQ ID NO: 73 - protein, 329 aa, Artificial Sequence
  variant of human IgG1f constant domain
ASTKGPSVFPLAPSSKSTSGGTAALGCLVKDYFPEPVTVSWNSGALTSGVHTFPAVLQSSGLYSLSSVVTVPSSSLGTQTYICNVNHKPSNTKVDKRVEPKSCDKTHTCPPCPAPELLGDDSVFLFPPKPKDTLMISRTPEVTCVVVDVSHEDGEVKFNWYVDGVEVHNAKTKPREEQYNSTYRVVSVLTVLHQDWLNGKEYKCKVSNKALPRPIEKTISKAKGQPREPQVYTLPPSREEMTKNQVSLTCLVKGFYPSDIAVEWESNGQPENNYKTTPPVLDSDGSFFLYSKLTVDKSRWQQGNVFSCSVMHEALHNHYTQKSLSLSPG

SEQ ID NO: 74 - protein, 329 aa, Artificial Sequence
  variant of human IgG1f constant domain
ASTKGPSVFPLAPSSKSTSGGTAALGCLVKDYFPEPVTVSWNSGALTSGVHTFPAVLQSSGLYSLSSVVTVPSSSLGTQTYICNVNHKPSNTKVDKRVEPKSCDKTHTCPPCPAPELLGDDSVFLFPPKPKDTLMISRTPEVTCVVVDVSHEEGEVKFNWYVDGVEVHNAKTKPREEQYNSTYRVVSVLTVLHQDWLNGKEYKCKVSNKALPRPIEKTISKAKGQPREPQVYTLPPSREEMTKNQVSLTCLVKGFYPSDIAVEWESNGQPENNYKTTPPVLDSDGSFFLYSKLTVDKSRWQQGNVFSCSVMHEALHNHYTQKSLSLSPG

SEQ ID NO: 75 - protein, 329 aa, Artificial Sequence
  variant of human IgG1f constant domain
ASTKGPSVFPLAPSSKSTSGGTAALGCLVKDYFPEPVTVSWNSGALTSGVHTFPAVLQSSGLYSLSSVVTVPSSSLGTQTYICNVNHKPSNTKVDKRVEPKSCDKTHTCPPCPAPELLGDDSVFLFPPKPKDTLMISRTPEVTCVVVDVSDEDGEVKFNWYVDGVEVHNAKTKPREEQYNSTYRVVSVLTVLHQDWLNGKEYKCKVSNKALPRPIEKTISKAKGQPREPQVYTLPPSREEMTKNQVSLTCLVKGFYPSDIAVEWESNGQPENNYKTTPPVLDSDGSFFLYSKLTVDKSRWQQGNVFSCSVMHEALHNHYTQKSLSLSPG

SEQ ID NO: 76 - protein, 329 aa, Artificial Sequence
  variant of human IgG1f constant domain
ASTKGPSVFPLAPSSKSTSGGTAALGCLVKDYFPEPVTVSWNSGALTSGVHTFPAVLQSSGLYSLSSVVTVPSSSLGTQTYICNVNHKPSNTKVDKRVEPKSCDKTHTCPPCPAPDLLGDDSVFLFPPKPKDTLMISRTPEVTCVVVDVSDEDGEVKFNWYVDGVEVHNAKTKPREEQYNSTYRVVSVLTVLHQDWLNGKEYKCKVSNKALPRPIEKTISKAKGQPREPQVYTLPPSREEMTKNQVSLTCLVKGFYPSDIAVEWESNGQPENNYKTTPPVLDSDGSFFLYSKLTVDKSRWQQGNVFSCSVMHEALHNHYTQKSLSLSPG

SEQ ID NO: 77 - protein, 107 aa, Homo sapiens [sequence omitted]

SEQ ID NO: 78 - protein, 17 aa, Homo sapiens
MRAWIFFLLCLAGRALA